European Patent Application EP 4 488 381 A1, published January 8, 2025. Title: MODIFIED DNA IDENTIFIER SEQUENCES FOR DNA MODIFICATION SCREENING. Applicant: ETH Zurich. Application EP. The sequence listing filed with the application follows.

SEQUENCE LISTING (10 sequences)

SEQ ID NO: 1 - DNA, 40 bp, synthetic construct
  source 1..40: mol_type = other DNA
  misc_feature 1: note = modified at the 5' end with an azido group
  misc_feature 40: note = labelled at the 3' end with biotin connected via a linker
  misc_feature 1..7: note = validation code nucleotide sequence, VC
  misc_feature 8..17: note = randomized index code nucleotide sequence, RIC
  misc_feature 18..40: note = annealing site nucleotide sequence, AS
tcaacaannnnnnnnnnagatcggaagagcgtcgtgtagg

SEQ ID NO: 2 - DNA, 40 bp, synthetic construct
  source 1..40: mol_type = other DNA
  misc_feature 1: note = modifed at the 5' end with an azido group
  misc_feature 1: note = validation code nucleotide sequence part 1, VCp1
  misc_feature 2..11: note = randomized index code nucleotide sequence, RIC
  misc_feature 12..17: note = validation code nucleotide sequence part 2, VCp2
  misc_feature 18..40: note = annealing site nucleotide sequence, AS
  misc_feature 40: note = labelled at the 3' end with biotin connected via a linker
tnnnnnnnnnncaacaaagatcggaagagcgtcgtgtagg

SEQ ID NO: 3 - DNA, 22 bp, synthetic construct
  source 1..22: mol_type = other DNA
cctacacgacgctcttccgatc

SEQ ID NO: 4 - DNA, 40 bp, synthetic construct; identical to SEQ ID NO: 2
  source 1..40: mol_type = other DNA
  misc_feature 1: note = modified at the 5' end with an azido group
  misc_feature 40: note = labelled at the 3' end with biotin connected via a triethylene glycol (TEG) linker

SEQ ID NO: 5 - DNA, 40 bp, synthetic construct; identical to SEQ ID NO: 1
  source 1..40: mol_type = other DNA
  misc_feature 1: note = modified at the 5' end with an azido group
  misc_feature 40: note = labelled at the 3' end with biotin connected via a triethylene glycol (TEG) linker

SEQ ID NO: 6 - DNA, 70 bp, synthetic construct
  source 1..70: mol_type = other DNA
  misc_feature 69^70: note = phosphothioester linkage
aatgatacggcgaccaccgagatctacactatagcctacactctttccctacacgacgctcttccgatct

SEQ ID NO: 7 - DNA, 66 bp, synthetic construct
  source 1..66: mol_type = other DNA
  misc_feature 65^66: note = phosphothioester linkage
caagcagaagacggcatacgagatcgagtaatgtgactggagttcagacgtgtgctcttccgatct

SEQ ID NO: 8 - DNA, 33 bp, synthetic construct
  source 1..33: mol_type = other DNA
  misc_feature 32^33: note = phosphothioester linkage
agacgtgtgctcttccgatctagaaggcctagt

SEQ ID NO: 9 - DNA, 32 bp, synthetic construct
  source 1..32: mol_type = other DNA
  misc_feature 1: note = 5'-phosphorylated
ctaggccttctaaggagatgttgatgtgctgc

SEQ ID NO: 10 - DNA, 22 bp, synthetic construct
  source 1..22: mol_type = other DNA
agacgtgtgctcttccgatcta